European Patent Application EP 4 324 851 A2, published February 21, 2024. Title: CHIMERIC ANTIGEN RECEPTORS WITH BCMA SPECIFICITY AND USES THEREOF. Applicant: Regeneron Pharmaceuticals, Inc. Application EP 1974907.2, filed July 18, 2019. The sequence listing filed with the application follows.

SEQUENCE LISTING (101 sequences)

SEQ ID NO: 1 - DNA, 366 bp, synthetic construct
  misc_feature 1..366: note = synthetic
  source 1..366: mol_type = other DNA
caggtgcagctggtggagtcggggggaggcgtggtccagcctgggaggtccctgagactctcctgtgcagcctctggattcaccttcagtacctatggcattcactgggtccgccaggctccaggcaaggggctggagtgggtggcagttatattacatgatggaagtagtaactactatgcagagtccgtgaagggccgattcatcatctccagagacaattccaagaacacactgtatctgcaaatgaacagcctgagagctgaggacacggctctatattactgtacgaaaaggtattcagaagcagctggcccaaattggttcgacccctggggccagggaaccctggtcaccgtctcctca

SEQ ID NO: 2 - protein, 122 aa, synthetic construct
  REGION 1..122: note = synthetic
QVQLVESGGGVVQPGRSLRLSCAASGFTFSTYGIHWVRQAPGKGLEWVAVILHDGSSNYYAESVKGRFIISRDNSKNTLYLQMNSLRAEDTALYYCTKRYSEAAGPNWFDPWGQGTLVTVSS

SEQ ID NO: 3 - DNA, 24 bp, synthetic construct
  misc_feature 1..24: note = synthetic
  source 1..24: mol_type = other DNA
ggattcaccttcagtacctatggc

SEQ ID NO: 4 - protein, 8 aa, synthetic construct
  REGION 1..8: note = synthetic
GFTFSTYG

SEQ ID NO: 5 - DNA, 24 bp, synthetic construct
  misc_feature 1..24: note = synthetic
  source 1..24: mol_type = other DNA
atattacatgatggaagtagtaac

SEQ ID NO: 6 - protein, 8 aa, synthetic construct
  REGION 1..8: note = synthetic
ILHDGSSN

SEQ ID NO: 7 - DNA, 45 bp, synthetic construct
  misc_feature 1..45: note = synthetic
  source 1..45: mol_type = other DNA
acgaaaaggtattcagaagcagctggcccaaattggttcgacccc

SEQ ID NO: 8 - protein, 15 aa, synthetic construct
  REGION 1..15: note = synthetic
TKRYSEAAGPNWFDP

SEQ ID NO: 9 - DNA, 321 bp, synthetic construct
  misc_feature 1..321: note = synthetic
  source 1..321: mol_type = other DNA
gacatccagatgacccagtctccatcctccgtgtctgcatctgtaggagacagagtcaccatcacttgtcgggcgagtcggggaattagcagctggttagcctggtatcagcagaagccagggaaagcccctaagctcctgatccatgctgcatccagtttgcaaagtggggtcccatcaaggttcagcggcagtggatctgggacagatttcactctcaccatcagcagcctgcagcctgaagattttgctacttactattgtcaacaggctatcagtttcccattcactttcggccctgggaccaaagtggatatcaaa

SEQ ID NO: 10 - protein, 107 aa, synthetic construct
  REGION 1..107: note = synthetic
DIQMTQSPSSVSASVGDRVTITCRASRGISSWLAWYQQKPGKAPKLLIHAASSLQSGVPSRFSGSGSGTDFTLTISSLQPEDFATYYCQQAISFPFTFGPGTKVDIK

SEQ ID NO: 11 - DNA, 18 bp, synthetic construct
  misc_feature 1..18: note = synthetic
  source 1..18: mol_type = other DNA
cggggaattagcagctgg

SEQ ID NO: 12 - protein, 6 aa, synthetic construct
  REGION 1..6: note = synthetic
RGISSW

SEQ ID NO: 13-14 - skipped (2 entries)

SEQ ID NO: 15 - DNA, 27 bp, synthetic construct
  misc_feature 1..27: note = synthetic
  source 1..27: mol_type = other DNA
caacaggctatcagtttcccattcact

SEQ ID NO: 16 - protein, 9 aa, synthetic construct
  REGION 1..9: note = synthetic
QQAISFPFT

SEQ ID NO: 17 - DNA, 360 bp, synthetic construct
  misc_feature 1..360: note = synthetic
  source 1..360: mol_type = other DNA
gaggtgcagctggtggagtctgggggaggcttggtacagcctggggggtccctgagactctcctgtgcagcctctggattcacctttagcagctatgtcatgagttgggtccgccaggctccagggaagggactggagtgggtctcagctattattggtagtggtggtagcacatattacgcagactccgtgaagggccggttcaccatctccagagacaattccaagaacacgctgtatctgcaaatgaacagcctgagagccgaggacacggccgtatattactgtgcgaaaagagccggggataactggaactggttcgacccctggggccagggaaccctggtcaccgtctcctca

SEQ ID NO: 18 - protein, 120 aa, synthetic construct
  REGION 1..120: note = synthetic
EVQLVESGGGLVQPGGSLRLSCAASGFTFSSYVMSWVRQAPGKGLEWVSAIIGSGGSTYYADSVKGRFTISRDNSKNTLYLQMNSLRAEDTAVYYCAKRAGDNWNWFDPWGQGTLVTVSS

SEQ ID NO: 19 - DNA, 24 bp, synthetic construct
  misc_feature 1..24: note = synthetic
  source 1..24: mol_type = other DNA
ggattcacctttagcagctatgtc

SEQ ID NO: 20 - protein, 8 aa, synthetic construct
  REGION 1..8: note = synthetic
GFTFSSYV

SEQ ID NO: 21 - DNA, 24 bp, synthetic construct
  misc_feature 1..24: note = synthetic
  source 1..24: mol_type = other DNA
attattggtagtggtggtagcaca

SEQ ID NO: 22 - protein, 8 aa, synthetic construct
  REGION 1..8: note = synthetic
IIGSGGST

SEQ ID NO: 23 - DNA, 39 bp, synthetic construct
  misc_feature 1..39: note = synthetic
  source 1..39: mol_type = other DNA
gcgaaaagagccggggataactggaactggttcgacccc

SEQ ID NO: 24 - protein, 13 aa, synthetic construct
  REGION 1..13: note = synthetic
AKRAGDNWNWFDP

SEQ ID NO: 25 - DNA, 321 bp, synthetic construct
  misc_feature 1..321: note = synthetic
  source 1..321: mol_type = other DNA
gacatccagatgacccagtctccatcttccgtgtctgcatctttaggagacagagtcaccatcacttgtcgggcgagtcagggtattagcagctggttagcctggtatcagcggaaaccagggaaagcccctaagctcctgatctatgctgcatccagtttgcaaagtggggtcccatcaaggttcagcggcagtggatctggggcggatttcactctcaccatcagcagcctgcagcctgaagattttgcaacttactattgtcaacaggctaaaagtgtcccattcactttcggccctgggaccaaagtggatatcaaa

SEQ ID NO: 26 - protein, 107 aa, synthetic construct
  REGION 1..107: note = synthetic
DIQMTQSPSSVSASLGDRVTITCRASQGISSWLAWYQRKPGKAPKLLIYAASSLQSGVPSRFSGSGSGADFTLTISSLQPEDFATYYCQQAKSVPFTFGPGTKVDIK

SEQ ID NO: 27 - DNA, 18 bp, synthetic construct
  misc_feature 1..18: note = synthetic
  source 1..18: mol_type = other DNA
cagggtattagcagctgg

SEQ ID NO: 28 - protein, 6 aa, synthetic construct
  REGION 1..6: note = synthetic
QGISSW

SEQ ID NO: 29-30 - skipped (2 entries)

SEQ ID NO: 31 - DNA, 27 bp, synthetic construct
  misc_feature 1..27: note = synthetic
  source 1..27: mol_type = other DNA
caacaggctaaaagtgtcccattcact

SEQ ID NO: 32 - protein, 9 aa, synthetic construct
  REGION 1..9: note = synthetic
QQAKSVPFT

SEQ ID NO: 33 - DNA, 351 bp, synthetic construct
  misc_feature 1..351: note = synthetic
  source 1..351: mol_type = other DNA
gaagtgcagctggtggagtctgggggaggcttggtacagcctggcaggtccctgagactctcctgtgcagcctctggattcacctttgatgattatgccatgcactgggtccggcaagctccagggaagggcctggagtgggtctcaggtatcagttggaatagtggtaacatgggatatgcggactctgtgaagggccgattcaccatctccagagacaacgccaagaactccctgttcctgcaaatgcacagtttgagagctgaggacacggccttttattactgtgcaaaagtccgtctaactgcctttgacttttggggccagggaaccctggtcaccgtctcctca

SEQ ID NO: 34 - protein, 117 aa, synthetic construct
  REGION 1..117: note = synthetic
EVQLVESGGGLVQPGRSLRLSCAASGFTFDDYAMHWVRQAPGKGLEWVSGISWNSGNMGYADSVKGRFTISRDNAKNSLFLQMHSLRAEDTAFYYCAKVRLTAFDFWGQGTLVTVSS

SEQ ID NO: 35 - DNA, 24 bp, synthetic construct
  misc_feature 1..24: note = synthetic
  source 1..24: mol_type = other DNA
ggattcacctttgatgattatgcc

SEQ ID NO: 36 - protein, 8 aa, synthetic construct
  REGION 1..8: note = synthetic
GFTFDDYA

SEQ ID NO: 37 - DNA, 24 bp, synthetic construct
  misc_feature 1..24: note = synthetic
  source 1..24: mol_type = other DNA
atcagttggaatagtggtaacatg

SEQ ID NO: 38 - protein, 8 aa, synthetic construct
  REGION 1..8: note = synthetic
ISWNSGNM

SEQ ID NO: 39 - DNA, 30 bp, synthetic construct
  misc_feature 1..30: note = synthetic
  source 1..30: mol_type = other DNA
gcaaaagtccgtctaactgcctttgacttt

SEQ ID NO: 40 - protein, 10 aa, synthetic construct
  REGION 1..10: note = synthetic
AKVRLTAFDF

SEQ ID NO: 41 - DNA, 321 bp, synthetic construct
  misc_feature 1..321: note = synthetic
  source 1..321: mol_type = other DNA
gacatccagatgacccagtctccatcctccctgtctgcatctgtaggagacagagtcaccatcacttgccggacaagtcagagcattggcaactatttaaattggtttcagcagaaaccagggaaagcccctaaactcctcatctatactgcatccagtttgcagaatggagtcccatcaaggttcactggcagtggatctgggacagatttcactctcaccatcagcagtctgcaacctgaggattttgtaatttactactgtcaacagagtttcagtaccccgtatacttttggccaggggaccaagctggagatcaaa

SEQ ID NO: 42 - protein, 107 aa, synthetic construct
  REGION 1..107: note = synthetic
DIQMTQSPSSLSASVGDRVTITCRTSQSIGNYLNWFQQKPGKAPKLLIYTASSLQNGVPSRFTGSGSGTDFTLTISSLQPEDFVIYYCQQSFSTPYTFGQGTKLEIK

SEQ ID NO: 43 - DNA, 18 bp, synthetic construct
  misc_feature 1..18: note = synthetic
  source 1..18: mol_type = other DNA
cagagcattggcaactat

SEQ ID NO: 44 - protein, 6 aa, synthetic construct
  REGION 1..6: note = synthetic
QSIGNY

SEQ ID NO: 45-46 - skipped (2 entries)

SEQ ID NO: 47 - DNA, 27 bp, synthetic construct
  misc_feature 1..27: note = synthetic
  source 1..27: mol_type = other DNA
caacagagtttcagtaccccgtatact

SEQ ID NO: 48 - protein, 9 aa, synthetic construct
  REGION 1..9: note = synthetic
QQSFSTPYT

SEQ ID NO: 49 - DNA, 354 bp, synthetic construct
  misc_feature 1..354: note = synthetic
  source 1..354: mol_type = other DNA
caggtgcagctggtggagtctgggggaggcttggtcaagcctggagggtccctgagactctcctgtgcagcctctggattcaccttcagtgactactacatcagctggatccgccaggctccagggaaggggctggagtgggtttcatacattagttctagtggtagttccataaagtacgcagactctgtgaagggccgattcaccatctccagggacaacgccaagaactcactgtatctgcaaatgaacagcctgagagccgaggacacggccgtatattactgtgcgagagagggagggaactacggtatggacgtctggggccaagggaccacggtcaccgtctcctca

SEQ ID NO: 50 - protein, 118 aa, synthetic construct
  REGION 1..118: note = synthetic
QVQLVESGGGLVKPGGSLRLSCAASGFTFSDYYISWIRQAPGKGLEWVSYISSSGSSIKYADSVKGRFTISRDNAKNSLYLQMNSLRAEDTAVYYCAREGGNYGMDVWGQGTTVTVSS

SEQ ID NO: 51 - DNA, 24 bp, synthetic construct
  misc_feature 1..24: note = synthetic
  source 1..24: mol_type = other DNA
ggattcaccttcagtgactactac

SEQ ID NO: 52 - protein, 8 aa, synthetic construct
  REGION 1..8: note = synthetic
GFTFSDYY

SEQ ID NO: 53 - DNA, 24 bp, synthetic construct
  misc_feature 1..24: note = synthetic
  source 1..24: mol_type = other DNA
attagttctagtggtagttccata

SEQ ID NO: 54 - protein, 8 aa, synthetic construct
  REGION 1..8: note = synthetic
ISSSGSSI

SEQ ID NO: 55 - DNA, 33 bp, synthetic construct
  misc_feature 1..33: note = synthetic
  source 1..33: mol_type = other DNA
gcgagagagggagggaactacggtatggacgtc

SEQ ID NO: 56 - protein, 11 aa, synthetic construct
  REGION 1..11: note = synthetic
AREGGNYGMDV

SEQ ID NO: 57 - DNA, 321 bp, synthetic construct
  misc_feature 1..321: note = synthetic
  source 1..321: mol_type = other DNA
gacatccagatgacccagtctccatcttccgtgtctgcatctgtaggagacagagtcaccatcacttgtcgggcgagtcagggtattaacaactggttagtctggtatcagcagaaaccagggaaagcccctaagctcctgatctatgctgcaaccagcttgcaaagtggggtcccatcaaggttcagcggcagtgggtctgggacagatttcactctcaccatcagcagcctgcagcctgaagattttgcaacttactattgtcaacaggctaacagtttccctcccacttttggccaggggaccaagctggagatcaaa

SEQ ID NO: 58 - protein, 107 aa, synthetic construct
  REGION 1..107: note = synthetic
DIQMTQSPSSVSASVGDRVTITCRASQGINNWLVWYQQKPGKAPKLLIYAATSLQSGVPSRFSGSGSGTDFTLTISSLQPEDFATYYCQQANSFPPTFGQGTKLEIK

SEQ ID NO: 59 - DNA, 18 bp, synthetic construct
  misc_feature 1..18: note = synthetic
  source 1..18: mol_type = other DNA
cagggtattaacaactgg

SEQ ID NO: 60 - protein, 6 aa, synthetic construct
  REGION 1..6: note = synthetic
QGINNW

SEQ ID NO: 61-62 - skipped (2 entries)

SEQ ID NO: 63 - DNA, 27 bp, synthetic construct
  misc_feature 1..27: note = synthetic
  source 1..27: mol_type = other DNA
caacaggctaacagtttccctcccact

SEQ ID NO: 64 - protein, 9 aa, synthetic construct
  REGION 1..9: note = synthetic
QQANSFPPT

SEQ ID NO: 65 - DNA, 375 bp, synthetic construct
  misc_feature 1..375: note = synthetic
  source 1..375: mol_type = other DNA
gaggtgcagctggtggagtctgggggaggcttggtccagcctggggggtccctgagactctcctgtgcagcctctggattcacctttagtaacttttggatgacctgggtccgccaggctccagggaaggggctggagtgggtggccaacatgaaccaagatggaagtgagaaatactatgtggactctgtgaagggccgattcaccatctccagagacaacgccaagagctcactgtatctgcaaatgaacagcctgagagccgaggacacggctgtgtattactgtgcgagagatcgggaatattgtattagtaccagctgctatgatgactttgactactggggccagggaaccctggtcaccgtctcctca

SEQ ID NO: 66 - protein, 125 aa, synthetic construct
  REGION 1..125: note = synthetic
EVQLVESGGGLVQPGGSLRLSCAASGFTFSNFWMTWVRQAPGKGLEWVANMNQDGSEKYYVDSVKGRFTISRDNAKSSLYLQMNSLRAEDTAVYYCARDREYCISTSCYDDFDYWGQGTLVTVSS

SEQ ID NO: 67 - DNA, 24 bp, synthetic construct
  misc_feature 1..24: note = synthetic
  source 1..24: mol_type = other DNA
ggattcacctttagtaacttttgg

SEQ ID NO: 68 - protein, 8 aa, synthetic construct
  REGION 1..8: note = synthetic
GFTFSNFW

SEQ ID NO: 69 - DNA, 24 bp, synthetic construct
  misc_feature 1..24: note = synthetic
  source 1..24: mol_type = other DNA
atgaaccaagatggaagtgagaaa

SEQ ID NO: 70 - protein, 8 aa, synthetic construct
  REGION 1..8: note = synthetic
MNQDGSEK

SEQ ID NO: 71 - DNA, 54 bp, synthetic construct
  misc_feature 1..54: note = synthetic
  source 1..54: mol_type = other DNA
gcgagagatcgggaatattgtattagtaccagctgctatgatgactttgactac

SEQ ID NO: 72 - protein, 18 aa, synthetic construct
  REGION 1..18: note = synthetic
ARDREYCISTSCYDDFDY

SEQ ID NO: 73 - DNA, 324 bp, synthetic construct
  misc_feature 1..324: note = synthetic
  source 1..324: mol_type = other DNA
gacatccagatgacccagtctccatcctccctgtctgcatctgtaggagacagagtcaccatcacttgccgggcaagtcagagcattagcagctatttaaattggtatcagcagaaaccagggaaagcccctaagctcctgatctatgctgcatccagtttgcatagtggggtcccatcaaggttcagtggcagtggatctgggacagatttcactctcaccatcagcagtctgcaacctgaagattttgcaacttactactgtcaacagagttacagtacccctccgatcaccttcggccaagggacacgactggagattaaa

SEQ ID NO: 74 - protein, 108 aa, synthetic construct
  REGION 1..108: note = synthetic
DIQMTQSPSSLSASVGDRVTITCRASQSISSYLNWYQQKPGKAPKLLIYAASSLHSGVPSRFSGSGSGTDFTLTISSLQPEDFATYYCQQSYSTPPITFGQGTRLEIK

SEQ ID NO: 75 - DNA, 18 bp, synthetic construct
  misc_feature 1..18: note = synthetic
  source 1..18: mol_type = other DNA
cagagcattagcagctat

SEQ ID NO: 76 - protein, 6 aa, synthetic construct
  REGION 1..6: note = synthetic
QSISSY

SEQ ID NO: 77-78 - skipped (2 entries)

SEQ ID NO: 79 - DNA, 30 bp, synthetic construct
  misc_feature 1..30: note = synthetic
  source 1..30: mol_type = other DNA
caacagagttacagtacccctccgatcacc

SEQ ID NO: 80 - protein, 10 aa, synthetic construct
  REGION 1..10: note = synthetic
QQSYSTPPIT

SEQ ID NO: 81 - DNA, 1404 bp, synthetic construct
  misc_feature 1..1404: note = BCMA 16711 (VL-VH) ScFv CAR-T (16711_VK_v2(human).(G4S)3 Linker.16711 VH.hCD8a hinge/TM.hCD137 (4-1BB).hCD3 zeta)
  source 1..1404: mol_type = other DNA
gacatccagatgacccagtctccatcctccgtgtctgcatctgtaggagacagagtcaccatcacttgtcgggcgagtcggggaattagcagctggttagcctggtatcagcagaagccagggaaagcccctaagctcctgatccatgctgcatccagtttgcaaagtggggtcccatcaaggttcagcggcagtggatctgggacagatttcactctcaccatcagcagcctgcagcctgaagattttgctacttactattgtcaacaggctatcagtttcccattcactttcggccctgggaccaaagtggatatcaaaggcggcggtggatctggaggcggtggaagcggtggcgggggaagtcaggtgcagctggtggagtcggggggaggcgtggtccagcctgggaggtccctgagactctcctgtgcagcctctggattcaccttcagtacctatggcattcactgggtccgccaggctccaggcaaggggctggagtgggtggcagttatattacatgatggaagtagtaactactatgcagagtccgtgaagggccgattcatcatctccagagacaattccaagaacacactgtatctgcaaatgaacagcctgagagctgaggacacggctctatattactgtacgaaaaggtattcagaagcagctggcccaaattggttcgacccctggggccagggaaccctggtcaccgtctcctcaactaccactcctgctccccgccccccaacacctgctccaactattgcatcccaaccactctccctcagacccgaagcttgtcgccccgccgccggaggtgctgttcacactagaggactcgattttgcttgcgacatttatatctgggccccacttgcaggtacttgcggagtattgctgctctcacttgttattactctttattgcaaacggggcagaaagaaactcctgtatatattcaaacaaccatttatgagaccagtacaaactactcaagaggaagatggctgtagctgccgatttccagaagaagaagaaggaggatgtgaactgagagtgaagttcagcaggagcgcagacgcccccgcgtacaagcagggccagaaccagctctataacgagctcaatctaggacgaagagaggagtacgatgttttggacaagagacgtggccgggaccctgagatggggggaaagccgagaaggaagaaccctcaggaaggcctgtacaatgaactgcagaaagataagatggcggaggcctacagtgagattgggatgaaaggcgagcgccggaggggcaaggggcacgatggcctttaccagggtctcagtacagccaccaaggacacctacgacgcccttcacatgcaggccctgccccctcgctaa

SEQ ID NO: 82 - protein, 467 aa, synthetic construct
  REGION 1..467: note = BCMA 16711 (VL-VH) ScFv CAR-T (16711_VK_v2(human).(G4S)3 Linker.16711 VH.hCD8a hinge/TM.hCD137 (4-1BB).hCD3 zeta)
DIQMTQSPSSVSASVGDRVTITCRASRGISSWLAWYQQKPGKAPKLLIHAASSLQSGVPSRFSGSGSGTDFTLTISSLQPEDFATYYCQQAISFPFTFGPGTKVDIKGGGGSGGGGSGGGGSQVQLVESGGGVVQPGRSLRLSCAASGFTFSTYGIHWVRQAPGKGLEWVAVILHDGSSNYYAESVKGRFIISRDNSKNTLYLQMNSLRAEDTALYYCTKRYSEAAGPNWFDPWGQGTLVTVSSTTTPAPRPPTPAPTIASQPLSLRPEACRPAAGGAVHTRGLDFACDIYIWAPLAGTCGVLLLSLVITLYCKRGRKKLLYIFKQPFMRPVQTTQEEDGCSCRFPEEEEGGCELRVKFSRSADAPAYKQGQNQLYNELNLGRREEYDVLDKRRGRDPEMGGKPRRKNPQEGLYNELQKDKMAEAYSEIGMKGERRRGKGHDGLYQGLSTATKDTYDALHMQALPPR

SEQ ID NO: 83 - DNA, 1398 bp, synthetic construct
  misc_feature 1..1398: note = BCMA 16716 (VL-VH) ScFv CAR-T (16716_VK(human).(G4S)3 Linker.16716_VH(human).hCD8a hinge/TM.hCD137 (4-1BB).hCD3 zeta)
  source 1..1398: mol_type = other DNA
gacatccagatgacccagtctccatcttccgtgtctgcatctttaggagacagagtcaccatcacttgtcgggcgagtcagggtattagcagctggttagcctggtatcagcggaaaccagggaaagcccctaagctcctgatctatgctgcatccagtttgcaaagtggggtcccatcaaggttcagcggcagtggatctggggcggatttcactctcaccatcagcagcctgcagcctgaagattttgcaacttactattgtcaacaggctaaaagtgtcccattcactttcggccctgggaccaaagtggatatcaaaggcggcggtggatctggaggcggtggaagcggtggcgggggaagtgaggtgcagctggtggagtctgggggaggcttggtacagcctggggggtccctgagactctcctgtgcagcctctggattcacctttagcagctatgtcatgagttgggtccgccaggctccagggaagggactggagtgggtctcagctattattggtagtggtggtagcacatattacgcagactccgtgaagggccggttcaccatctccagagacaattccaagaacacgctgtatctgcaaatgaacagcctgagagccgaggacacggccgtatattactgtgcgaaaagagccggggataactggaactggttcgacccctggggccagggaaccctggtcaccgtctcctcaactaccactcctgctccccgccccccaacacctgctccaactattgcatcccaaccactctccctcagacccgaagcttgtcgccccgccgccggaggtgctgttcacactagaggactcgattttgcttgcgacatttatatctgggccccacttgcaggtacttgcggagtattgctgctctcacttgttattactctttattgcaaacggggcagaaagaaactcctgtatatattcaaacaaccatttatgagaccagtacaaactactcaagaggaagatggctgtagctgccgatttccagaagaagaagaaggaggatgtgaactgagagtgaagttcagcaggagcgcagacgcccccgcgtacaagcagggccagaaccagctctataacgagctcaatctaggacgaagagaggagtacgatgttttggacaagagacgtggccgggaccctgagatggggggaaagccgagaaggaagaaccctcaggaaggcctgtacaatgaactgcagaaagataagatggcggaggcctacagtgagattgggatgaaaggcgagcgccggaggggcaaggggcacgatggcctttaccagggtctcagtacagccaccaaggacacctacgacgcccttcacatgcaggccctgccccctcgctaa

SEQ ID NO: 84 - protein, 465 aa, synthetic construct
  REGION 1..465: note = BCMA 16716 (VL-VH) ScFv CAR-T (16716_VK(human).(G4S)3 Linker.16716_VH(human).hCD8a hinge/TM.hCD137 (4-1BB).hCD3 zeta)
DIQMTQSPSSVSASLGDRVTITCRASQGISSWLAWYQRKPGKAPKLLIYAASSLQSGVPSRFSGSGSGADFTLTISSLQPEDFATYYCQQAKSVPFTFGPGTKVDIKGGGGSGGGGSGGGGSEVQLVESGGGLVQPGGSLRLSCAASGFTFSSYVMSWVRQAPGKGLEWVSAIIGSGGSTYYADSVKGRFTISRDNSKNTLYLQMNSLRAEDTAVYYCAKRAGDNWNWFDPWGQGTLVTVSSTTTPAPRPPTPAPTIASQPLSLRPEACRPAAGGAVHTRGLDFACDIYIWAPLAGTCGVLLLSLVITLYCKRGRKKLLYIFKQPFMRPVQTTQEEDGCSCRFPEEEEGGCELRVKFSRSADAPAYKQGQNQLYNELNLGRREEYDVLDKRRGRDPEMGGKPRRKNPQEGLYNELQKDKMAEAYSEIGMKGERRRGKGHDGLYQGLSTATKDTYDALHMQALPPR

SEQ ID NO: 85 - DNA, 1389 bp, synthetic construct
  misc_feature 1..1389: note = BCMA 16732 (VL-VH) ScFv CAR-T (16732_VK_v2(human).(G4S)3 Linker.16732_VH(human).hCD8a hinge/TM.hCD137 (4-1BB).hCD3 zeta)
  source 1..1389: mol_type = other DNA
gacatccagatgacccagtctccatcctccctgtctgcatctgtaggagacagagtcaccatcacttgccggacaagtcagagcattggcaactatttaaattggtttcagcagaaaccagggaaagcccctaaactcctcatctatactgcatccagtttgcagaatggagtcccatcaaggttcactggcagtggatctgggacagatttcactctcaccatcagcagtctgcaacctgaggattttgtaatttactactgtcaacagagtttcagtaccccgtatacttttggccaggggaccaagctggagatcaaaggcggcggtggatctggaggcggtggaagcggtggcgggggaagtgaagtgcagctggtggagtctgggggaggcttggtacagcctggcaggtccctgagactctcctgtgcagcctctggattcacctttgatgattatgccatgcactgggtccggcaagctccagggaagggcctggagtgggtctcaggtatcagttggaatagtggtaacatgggatatgcggactctgtgaagggccgattcaccatctccagagacaacgccaagaactccctgttcctgcaaatgcacagtttgagagctgaggacacggccttttattactgtgcaaaagtccgtctaactgcctttgacttttggggccagggaaccctggtcaccgtctcctcaactaccactcctgctccccgccccccaacacctgctccaactattgcatcccaaccactctccctcagacccgaagcttgtcgccccgccgccggaggtgctgttcacactagaggactcgattttgcttgcgacatttatatctgggccccacttgcaggtacttgcggagtattgctgctctcacttgttattactctttattgcaaacggggcagaaagaaactcctgtatatattcaaacaaccatttatgagaccagtacaaactactcaagaggaagatggctgtagctgccgatttccagaagaagaagaaggaggatgtgaactgagagtgaagttcagcaggagcgcagacgcccccgcgtacaagcagggccagaaccagctctataacgagctcaatctaggacgaagagaggagtacgatgttttggacaagagacgtggccgggaccctgagatggggggaaagccgagaaggaagaaccctcaggaaggcctgtacaatgaactgcagaaagataagatggcggaggcctacagtgagattgggatgaaaggcgagcgccggaggggcaaggggcacgatggcctttaccagggtctcagtacagccaccaaggacacctacgacgcccttcacatgcaggccctgccccctcgctaa

SEQ ID NO: 86 - protein, 462 aa, synthetic construct
  REGION 1..462: note = BCMA 16732 (VL-VH) ScFv CAR-T (16732_VK_v2(human).(G4S)3 Linker.16732_VH(human).hCD8a hinge/TM.hCD137 (4-1BB).hCD3 zeta)
DIQMTQSPSSLSASVGDRVTITCRTSQSIGNYLNWFQQKPGKAPKLLIYTASSLQNGVPSRFTGSGSGTDFTLTISSLQPEDFVIYYCQQSFSTPYTFGQGTKLEIKGGGGSGGGGSGGGGSEVQLVESGGGLVQPGRSLRLSCAASGFTFDDYAMHWVRQAPGKGLEWVSGISWNSGNMGYADSVKGRFTISRDNAKNSLFLQMHSLRAEDTAFYYCAKVRLTAFDFWGQGTLVTVSSTTTPAPRPPTPAPTIASQPLSLRPEACRPAAGGAVHTRGLDFACDIYIWAPLAGTCGVLLLSLVITLYCKRGRKKLLYIFKQPFMRPVQTTQEEDGCSCRFPEEEEGGCELRVKFSRSADAPAYKQGQNQLYNELNLGRREEYDVLDKRRGRDPEMGGKPRRKNPQEGLYNELQKDKMAEAYSEIGMKGERRRGKGHDGLYQGLSTATKDTYDALHMQALPPR

SEQ ID NO: 87 - DNA, 1392 bp, synthetic construct
  misc_feature 1..1392: note = BCMA 16747 (VL-VH) ScFv CAR-T (16747_VK(human).(G4S)3 Linker.16747_VH(human).hCD8a hinge/TM.hCD137 (4-1BB).hCD3 zeta)
  source 1..1392: mol_type = other DNA
gacatccagatgacccagtctccatcttccgtgtctgcatctgtaggagacagagtcaccatcacttgtcgggcgagtcagggtattaacaactggttagtctggtatcagcagaaaccagggaaagcccctaagctcctgatctatgctgcaaccagcttgcaaagtggggtcccatcaaggttcagcggcagtgggtctgggacagatttcactctcaccatcagcagcctgcagcctgaagattttgcaacttactattgtcaacaggctaacagtttccctcccacttttggccaggggaccaagctggagatcaaaggcggcggtggatctggaggcggtggaagcggtggcgggggaagtcaggtgcagctggtggagtctgggggaggcttggtcaagcctggagggtccctgagactctcctgtgcagcctctggattcaccttcagtgactactacatcagctggatccgccaggctccagggaaggggctggagtgggtttcatacattagttctagtggtagttccataaagtacgcagactctgtgaagggccgattcaccatctccagggacaacgccaagaactcactgtatctgcaaatgaacagcctgagagccgaggacacggccgtatattactgtgcgagagagggagggaactacggtatggacgtctggggccaagggaccacggtcaccgtctcctcaactaccactcctgctccccgccccccaacacctgctccaactattgcatcccaaccactctccctcagacccgaagcttgtcgccccgccgccggaggtgctgttcacactagaggactcgattttgcttgcgacatttatatctgggccccacttgcaggtacttgcggagtattgctgctctcacttgttattactctttattgcaaacggggcagaaagaaactcctgtatatattcaaacaaccatttatgagaccagtacaaactactcaagaggaagatggctgtagctgccgatttccagaagaagaagaaggaggatgtgaactgagagtgaagttcagcaggagcgcagacgcccccgcgtacaagcagggccagaaccagctctataacgagctcaatctaggacgaagagaggagtacgatgttttggacaagagacgtggccgggaccctgagatggggggaaagccgagaaggaagaaccctcaggaaggcctgtacaatgaactgcagaaagataagatggcggaggcctacagtgagattgggatgaaaggcgagcgccggaggggcaaggggcacgatggcctttaccagggtctcagtacagccaccaaggacacctacgacgcccttcacatgcaggccctgccccctcgctaa

SEQ ID NO: 88 - protein, 463 aa, synthetic construct
  REGION 1..463: note = BCMA 16747 (VL-VH) ScFv CAR-T (16747_VK(human).(G4S)3 Linker.16747_VH(human).hCD8a hinge/TM.hCD137 (4-1BB).hCD3 zeta)
DIQMTQSPSSVSASVGDRVTITCRASQGINNWLVWYQQKPGKAPKLLIYAATSLQSGVPSRFSGSGSGTDFTLTISSLQPEDFATYYCQQANSFPPTFGQGTKLEIKGGGGSGGGGSGGGGSQVQLVESGGGLVKPGGSLRLSCAASGFTFSDYYISWIRQAPGKGLEWVSYISSSGSSIKYADSVKGRFTISRDNAKNSLYLQMNSLRAEDTAVYYCAREGGNYGMDVWGQGTTVTVSSTTTPAPRPPTPAPTIASQPLSLRPEACRPAAGGAVHTRGLDFACDIYIWAPLAGTCGVLLLSLVITLYCKRGRKKLLYIFKQPFMRPVQTTQEEDGCSCRFPEEEEGGCELRVKFSRSADAPAYKQGQNQLYNELNLGRREEYDVLDKRRGRDPEMGGKPRRKNPQEGLYNELQKDKMAEAYSEIGMKGERRRGKGHDGLYQGLSTATKDTYDALHMQALPPR

SEQ ID NO: 89 - DNA, 1431 bp, synthetic construct
  misc_feature 1..1431: note = BCMA 21581 (VL-VH) ScFv CAR-T (21581 VK(human).(G4S)3 Linker.21581 VH(human).G4S Linker_v2.hCD8a hinge/TM.hCD137 (4-1BB).hCD3 zeta)
  source 1..1431: mol_type = other DNA
gacatccagatgacccagtctccatcctccctgtctgcatctgtaggagacagagtcaccatcacttgccgggcaagtcagagcattagcagctatttaaattggtatcagcagaaaccagggaaagcccctaagctcctgatctatgctgcatccagtttgcatagtggggtcccatcaaggttcagtggcagtggatctgggacagatttcactctcaccatcagcagtctgcaacctgaagattttgcaacttactactgtcaacagagttacagtacccctccgatcaccttcggccaagggacacgactggagattaaaggcggcggtggatctggaggcggtggaagcggtggcgggggaagtgaggtgcagctggtggagtctgggggaggcttggtccagcctggggggtccctgagactctcctgtgcagcctctggattcacctttagtaacttttggatgacctgggtccgccaggctccagggaaggggctggagtgggtggccaacatgaaccaagatggaagtgagaaatactatgtggactctgtgaagggccgattcaccatctccagagacaacgccaagagctcactgtatctgcaaatgaacagcctgagagccgaggacacggctgtgtattactgtgcgagagatcgggaatattgtattagtaccagctgctatgatgactttgactactggggccagggaaccctggtcaccgtctcctcaggaggcggaggcagcactaccactcctgctccccgccccccaacacctgctccaactattgcatcccaaccactctccctcagacccgaagcttgtcgccccgccgccggaggtgctgttcacactagaggactcgattttgcttgcgacatttatatctgggccccacttgcaggtacttgcggagtattgctgctctcacttgttattactctttattgcaaacggggcagaaagaaactcctgtatatattcaaacaaccatttatgagaccagtacaaactactcaagaggaagatggctgtagctgccgatttccagaagaagaagaaggaggatgtgaactgagagtgaagttcagcaggagcgcagacgcccccgcgtacaagcagggccagaaccagctctataacgagctcaatctaggacgaagagaggagtacgatgttttggacaagagacgtggccgggaccctgagatggggggaaagccgagaaggaagaaccctcaggaaggcctgtacaatgaactgcagaaagataagatggcggaggcctacagtgagattgggatgaaaggcgagcgccggaggggcaaggggcacgatggcctttaccagggtctcagtacagccaccaaggacacctacgacgcccttcacatgcaggccctgccccctcgctaa

SEQ ID NO: 90 - protein, 476 aa, synthetic construct
  REGION 1..476: note = BCMA 21581 (VL-VH) ScFv CAR-T (21581 VK(human).(G4S)3 Linker.21581 VH(human).G4S Linker_v2.hCD8a hinge/TM.hCD137 (4-1BB).hCD3 zeta)
DIQMTQSPSSLSASVGDRVTITCRASQSISSYLNWYQQKPGKAPKLLIYAASSLHSGVPSRFSGSGSGTDFTLTISSLQPEDFATYYCQQSYSTPPITFGQGTRLEIKGGGGSGGGGSGGGGSEVQLVESGGGLVQPGGSLRLSCAASGFTFSNFWMTWVRQAPGKGLEWVANMNQDGSEKYYVDSVKGRFTISRDNAKSSLYLQMNSLRAEDTAVYYCARDREYCISTSCYDDFDYWGQGTLVTVSSGGGGSTTTPAPRPPTPAPTIASQPLSLRPEACRPAAGGAVHTRGLDFACDIYIWAPLAGTCGVLLLSLVITLYCKRGRKKLLYIFKQPFMRPVQTTQEEDGCSCRFPEEEEGGCELRVKFSRSADAPAYKQGQNQLYNELNLGRREEYDVLDKRRGRDPEMGGKPRRKNPQEGLYNELQKDKMAEAYSEIGMKGERRRGKGHDGLYQGLSTATKDTYDALHMQALPPR

SEQ ID NO: 91 - DNA, 1437 bp, synthetic construct
  misc_feature 1..1437: note = HLA-A2/HPV16E7(11-19) 17363 ScFv (VL-VH) CAR-T (Irrelevant Control) (17363_ULC-VK(1)(human).G4Sx3_4.17363_VH(human). G4S_V2.hCD8a hinge/TM.hCD137 (4-1BB).hCD3 zeta)
  source 1..1437: mol_type = other DNA
gacatccagatgacccagtctccatcctccctgtctgcatctgtaggagacagagtcaccatcacttgccgggcaagtcagagcattagcagctatttaaattggtatcaacagaaaccagggaaagcccctaagctcctgatctatgctgtttccattttgcaaagtggggtcccatcaaggttcagtggcagtggatctgggacagatttcactctcaccatcaactctctgcaacctgaagattttgcaacttactcctgtcaacagacttacagtacccctccgatcaccttcggccaagggacacgactggagattaaaggtggaggcggtagtggcggaggcggaagtggtggaggaggctcagaggtgcagctgttggagtctgggggaggcttggtacaacctggggggtccctgagactctcctgtgcagcctctggattcacctttagcagttatgccatgacctgggtccgccaggctccagggatgggactggagtgggtctcagttattagtggtagtggtagtgaaacatactacgcagactccgtgaagggccggttcaccatctccagagacaattccaaaaacacactgtatctgcaaatgaacagcctgagagccgaagacacggccgtatattactgtgtgaaagattcttcgtataggagctcgtcgagggcctactactactacggaatggacgtctggggcctagggaccacggtcaccgtctcctcaggaggtggtggaagtactaccactcctgctccccgccccccaacacctgctccaactattgcatcccaaccactctccctcagacccgaagcttgtcgccccgccgccggaggtgctgttcacactagaggactcgattttgcttgcgacatttatatctgggccccacttgcaggtacttgcggagtattgctgctctcacttgttattactctttattgcaaacggggcagaaagaaactcctgtatatattcaaacaaccatttatgagaccagtacaaactactcaagaggaagatggctgtagctgccgatttccagaagaagaagaaggaggatgtgaactgagagtgaagttcagcaggagcgcagacgcccccgcgtacaagcagggccagaaccagctctataacgagctcaatctaggacgaagagaggagtacgatgttttggacaagagacgtggccgggaccctgagatggggggaaagccgagaaggaagaaccctcaggaaggcctgtacaatgaactgcagaaagataagatggcggaggcctacagtgagattgggatgaaaggcgagcgccggaggggcaaggggcacgatggcctttaccagggtctcagtacagccaccaaggacacctacgacgcccttcacatgcaggccctgccccctcgctaa

SEQ ID NO: 92 - protein, 478 aa, synthetic construct
  REGION 1..478: note = HLA-A2/HPV16E7(11-19) 17363 ScFv (VL-VH) CAR-T (Irrelevant Control) (17363_ULC-VK(1)(human).G4Sx3_4.17363_VH(human). G4S_V2.hCD8a hinge/TM.hCD137 (4-1BB).hCD3 zeta)
DIQMTQSPSSLSASVGDRVTITCRASQSISSYLNWYQQKPGKAPKLLIYAVSILQSGVPSRFSGSGSGTDFTLTINSLQPEDFATYSCQQTYSTPPITFGQGTRLEIKGGGGSGGGGSGGGGSEVQLLESGGGLVQPGGSLRLSCAASGFTFSSYAMTWVRQAPGMGLEWVSVISGSGSETYYADSVKGRFTISRDNSKNTLYLQMNSLRAEDTAVYYCVKDSSYRSSSRAYYYYGMDVWGLGTTVTVSSGGGGSTTTPAPRPPTPAPTIASQPLSLRPEACRPAAGGAVHTRGLDFACDIYIWAPLAGTCGVLLLSLVITLYCKRGRKKLLYIFKQPFMRPVQTTQEEDGCSCRFPEEEEGGCELRVKFSRSADAPAYKQGQNQLYNELNLGRREEYDVLDKRRGRDPEMGGKPRRKNPQEGLYNELQKDKMAEAYSEIGMKGERRRGKGHDGLYQGLSTATKDTYDALHMQALPPR

SEQ ID NO: 93 - protein, 5 aa, synthetic construct
  REGION 1..5: note = linker
GGGGS

SEQ ID NO: 94 - protein, 10 aa, synthetic construct
  REGION 1..10: note = linker
GGGGSGGGGS

SEQ ID NO: 95 - protein, 15 aa, synthetic construct
  REGION 1..15: note = linker
GGGGSGGGGSGGGGS

SEQ ID NO: 96 - protein, 18 aa, synthetic construct
  REGION 1..18: note = linker
GSTSGSGKPGSGEGSTKG

SEQ ID NO: 97 - protein, 45 aa, synthetic construct
  REGION 1..45: note = hinge
TTTPAPRPPTPAPTIASQPLSLRPEACRPAAGGAVHTRGLDFACD

SEQ ID NO: 98 - protein, 24 aa, synthetic construct
  REGION 1..24: note = TM domain
IYIWAPLAGTCGVLLLSLVITLYC

SEQ ID NO: 99 - protein, 42 aa, synthetic construct
  REGION 1..42: note = 4-1BB
KRGRKKLLYIFKQPFMRPVQTTQEEDGCSCRFPEEEEGGCEL

SEQ ID NO: 100 - protein, 112 aa, synthetic construct
  REGION 1..112: note = cd3-Zeta
RVKFSRSADAPAYKQGQNQLYNELNLGRREEYDVLDKRRGRDPEMGGKPRRKNPQEGLYNELQKDKMAEAYSEIGMKGERRRGKGHDGLYQGLSTATKDTYDALHMQALPPR

SEQ ID NO: 101 - protein, 184 aa, synthetic construct
  REGION 1..184: note = human BCMA (TNFRSF17) Protein NP_001183.2
MLQMAGQCSQNEYFDSLLHACIPCQLRCSSNTPPLTCQRYCNASVTNSVKGTNAILWTCLGLSLIISLAVFVLMFLLRKINSEPLKDEFKNTGSGLLGMANIDLEKSRTGDEIILPRGLEYTVEECTCEDCIKSKPKVDSDHCFPLPAMEEGATILVTTKTNDYCKSLPAALSATEIEKSISAR